European Patent Application EP 4 650 368 A1, published November 19, 2025. Title: Tetravalent agonists of erythropoietin receptor. Applicant: EPOK THERAPEUTICS INC. The sequence listing filed with the application follows.

SEQUENCE LISTING (32 sequences)

SEQ ID NO: 1 - protein, 5 aa, synthetic construct
SVSSA

SEQ ID NO: 2 - protein, 7 aa, synthetic construct
SASSLYS

SEQ ID NO: 3 - protein, 6 aa, synthetic construct
SSXFLI

SEQ ID NO: 4 - protein, 6 aa, synthetic construct
LDSYYM

SEQ ID NO: 5 - protein, 10 aa, synthetic construct
SIAPYHGYTY

SEQ ID NO: 6 - protein, 6 aa, synthetic construct
HGYGAL

SEQ ID NO: 7 - protein, 5 aa, synthetic construct
GGGGG

SEQ ID NO: 8 - protein, 9 aa, synthetic construct
IKGGGGGEV

SEQ ID NO: 9 - protein, 9 aa, synthetic construct
LKVLSRGVV

SEQ ID NO: 10 - protein, 9 aa, synthetic construct
ISARAGSLV

SEQ ID NO: 11 - protein, 9 aa, synthetic construct
SKSRAGGEV

SEQ ID NO: 12 - protein, 9 aa, synthetic construct
LKGGRGGKV

SEQ ID NO: 13 - protein, 9 aa, synthetic construct
NKGGGGAKV

SEQ ID NO: 14 - protein, 9 aa, synthetic construct
IKGSSRDDI

SEQ ID NO: 15 - protein, 9 aa, synthetic construct
MKHAGRGGV

SEQ ID NO: 16 - protein, 9 aa, synthetic construct
SKGGGGGEV

SEQ ID NO: 17 - protein, 9 aa, synthetic construct
MKHAGRGGV

SEQ ID NO: 18 - protein, 9 aa, synthetic construct
LECSDCSGI

SEQ ID NO: 19 - protein, 330 aa, synthetic construct [sequence omitted]

SEQ ID NO: 20 - protein, 224 aa, synthetic construct
DIQMTQSPSSLSASVGDRVTITCRASQSVSSAVAWYQQKPGKAPKLLIYSASSLYSGVPSRFSGSRSGTDFTLTISSLQPEDFATYYCQQSSNFLITFGQGTKVEIKEVQLVESGGGLVQPGGSLRLSCAASGFTLDSYYMHWVRQAPGKGLEWVASIAPYHGYTYYADSVKGRFTISADTSKNTAYLQMNSLRAEDTAVYYCARHGYGALDYWGQGTLVTVSS

SEQ ID NO: 21 - protein, 225 aa, synthetic construct
DIQMTQSPSSLSASVGDRVTITCRASQSVSSAVAWYQQKPGKAPKLLIYSASSLYSGVPSRFSGSRSGTDFTLTISSLQPEDFATYYCQQSSNFLITFGQGTKVEIKGEVQLVESGGGLVQPGGSLRLSCAASGFTLDSYYMHWVRQAPGKGLEWVASIAPYHGYTYYADSVKGRFTISADTSKNTAYLQMNSLRAEDTAVYYCARHGYGALDYWGQGTLVTVSS

SEQ ID NO: 22 - protein, 226 aa, synthetic construct
DIQMTQSPSSLSASVGDRVTITCRASQSVSSAVAWYQQKPGKAPKLLIYSASSLYSGVPSRFSGSRSGTDFTLTISSLQPEDFATYYCQQSSNFLITFGQGTKVEIKGGEVQLVESGGGLVQPGGSLRLSCAASGFTLDSYYMHWVRQAPGKGLEWVASIAPYHGYTYYADSVKGRFTISADTSKNTAYLQMNSLRAEDTAVYYCARHGYGALDYWGQGTLVTVSS

SEQ ID NO: 23 - protein, 466 aa, synthetic construct
DIQMTQSPSSLSASVGDRVTITCRASQSVSSAVAWYQQKPGKAPKLLIYSASSLYSGVPSRFSGSRSGTDFTLTISSLQPEDFATYYCQQSSNFLITFGQGTKVEIKEVQLVESGGGLVQPGGSLRLSCAASGFTLDSYYMHWVRQAPGKGLEWVASIAPYHGYTYYADSVKGRFTISADTSKNTAYLQMNSLRAEDTAVYYCARHGYGALDYWGQGTLVTVSSGGGGSGGGGSEPKSSDKTHTCPPCPAPEAAGGPSVFLFPPKPKDTLMISRTPEVTCVVVDVSHEDPEVKFNWYVDGVEVHNAKTKPREEQYNSTYRVVSVLTVLHQDWLNGKEYKCKVSNKALPASIEKTISKAKGQPREPQVYTLPPSREEMTKNQVSLTCLVKGFYPSDIAVEWESNGQPENNYKTTPPVLDSDGSFFLYSKLTVDKSRWQQGNVFSCSVMHEALHNHYTQKSLSLSPGK

SEQ ID NO: 24 - protein, 467 aa, synthetic construct
DIQMTQSPSSLSASVGDRVTITCRASQSVSSAVAWYQQKPGKAPKLLIYSASSLYSGVPSRFSGSRSGTDFTLTISSLQPEDFATYYCQQSSNFLITFGQGTKVEIKGEVQLVESGGGLVQPGGSLRLSCAASGFTLDSYYMHWVRQAPGKGLEWVASIAPYHGYTYYADSVKGRFTISADTSKNTAYLQMNSLRAEDTAVYYCARHGYGALDYWGQGTLVTVSSGGGGSGGGGSEPKSSDKTHTCPPCPAPEAAGGPSVFLFPPKPKDTLMISRTPEVTCVVVDVSHEDPEVKFNWYVDGVEVHNAKTKPREEQYNSTYRVVSVLTVLHQDWLNGKEYKCKVSNKALPASIEKTISKAKGQPREPQVYTLPPSREEMTKNQVSLTCLVKGFYPSDIAVEWESNGQPENNYKTTPPVLDSDGSFFLYSKLTVDKSRWQQGNVFSCSVMHEALHNHYTQKSLSLSPGK

SEQ ID NO: 25 - protein, 468 aa, synthetic construct
DIQMTQSPSSLSASVGDRVTITCRASQSVSSAVAWYQQKPGKAPKLLIYSASSLYSGVPSRFSGSRSGTDFTLTISSLQPEDFATYYCQQSSNFLITFGQGTKVEIKGGEVQLVESGGGLVQPGGSLRLSCAASGFTLDSYYMHWVRQAPGKGLEWVASIAPYHGYTYYADSVKGRFTISADTSKNTAYLQMNSLRAEDTAVYYCARHGYGALDYWGQGTLVTVSSGGGGSGGGGSEPKSSDKTHTCPPCPAPEAAGGPSVFLFPPKPKDTLMISRTPEVTCVVVDVSHEDPEVKFNWYVDGVEVHNAKTKPREEQYNSTYRVVSVLTVLHQDWLNGKEYKCKVSNKALPASIEKTISKAKGQPREPQVYTLPPSREEMTKNQVSLTCLVKGFYPSDIAVEWESNGQPENNYKTTPPVLDSDGSFFLYSKLTVDKSRWQQGNVFSCSVMHEALHNHYTQKSLSLSPGK

SEQ ID NO: 26 - protein, 720 aa, synthetic construct
DIQMTQSPSSLSASVGDRVTITCRASQSVSSAVAWYQQKPGKAPKLLIYSASSLYSGVPSRFSGSRSGTDFTLTISSLQPEDFATYYCQQSSQFLITFGQGTKVEIKGGGGGEVQLVESGGGLVQPGGSLRLSCAASGFTLDSYYMHWVRQAPGKGLEWVASIAPYHGYTYYADSVKGRFTISADTSKNTAYLQMNSLRAEDTAVYYCARHGYGALDYWGQGTLVTVSSGGGGSGGGGSEPKSSDKTHTCPPCPAPEAAGGPSVFLFPPKPKDTLMISRTPEVTCVVVDVSHEDPEVKFNWYVDGVEVHNAKTKPREEQYNSTYRVVSVLTVLHQDWLNGKEYKCKVSNKALPASIEKTISKAKGQPREPQVYTLPPSREEMTKNQVSLTCLVKGFYPSDIAVEWESNGQPENNYKTTPPVLDSDGSFFLYSKLTVDKSRWQQGNVFSCSVMHEALHNHYTQKSLSLSPGKGGGGSGGGGSGGGGSGGGGSDIQMTQSPSSLSASVGDRVTITCRASQSVSSAVAWYQQKPGKAPKLLIYSASSLYSGVPSRFSGSRSGTDFTLTISSLQPEDFATYYCQQSSQFLITFGQGTKVEIKGGGGGEVQLVESGGGLVQPGGSLRLSCAASGFTLDSYYMHWVRQAPGKGLEWVASIAPYHGYTYYADSVKGRFTISADTSKNTAYLQMNSLRAEDTAVYYCARHGYGALDYWGQGTLVTVSS

SEQ ID NO: 27 - protein, 716 aa, synthetic construct
DIQMTQSPSSLSASVGDRVTITCRASQSVSSAVAWYQQKPGKAPKLLIYSASSLYSGVPSRFSGSRSGTDFTLTISSLQPEDFATYYCQQSSQFLITFGQGTKVEIKGGGGGEVQLVESGGGLVQPGGSLRLSCAASGFTLDSYYMHWVRQAPGKGLEWVASIAPYHGYTYYADSVKGRFTISADTSKNTAYLQMNSLRAEDTAVYYCARHGYGALDYWGQGTLVTVSSGGGGSGGGGSEPKSSDKTHTCPPCPAPEAAGGPSVFLFPPKPKDTLMISRTPEVTCVVVDVSHEDPEVKFNWYVDGVEVHNAKTKPREEQYNSTYRVVSVLTVLHQDWLNGKEYKCKVSNKALPASIEKTISKAKGQPREPQVYTLPPSREEMTKNQVSLTCLVKGFYPSDIAVEWESNGQPENNYKTTPPVLDSDGSFFLYSKLTVDKSRWQQGNVFSCSVMHEALHNHYTQKSLSLSPGKGGGGSGGGGSGGGGSGGGGSEVQLVESGGGLVQPGGSLRLSCAASGFTLDSYYMHWVRQAPGKGLEWVASIAPYHGYTYYADSVKGRFTISADTSKNTAYLQMNSLRAEDTAVYYCARHGYGALDYWGQGTLVTVSSASTKGPSVFPLAPSSKSTSGGTAALGCLVKDYFPEPVTVSWNSGALTSGVHTFPAVLQSSGLYSLSSVVTVPSSSLGTQTYICNVNHKPSNTKVDKKVEPKSCDKTHT

SEQ ID NO: 28 - protein, 214 aa, synthetic construct
DIQMTQSPSSLSASVGDRVTITCRASQSVSSAVAWYQQKPGKAPKLLIYSASSLYSGVPSRFSGSRSGTDFTLTISSLQPEDFATYYCQQSSQFLITFGQGTKVEIKRTVAAPSVFIFPPSDEQLKSGTASVVCLLNNFYPREAKVQWKVDNALQSGNSQESVTEQDSKDSTYSLSSTLTLSKADYEKHKVYACEVTHQGLSSPVTKSFNRGEC

SEQ ID NO: 29 - protein, 696 aa, synthetic construct
EVQLVESGGGLVQPGGSLRLSCAASGFTLDSYYMHWVRQAPGKGLEWVASIAPYHGYTYYADSVKGRFTISADTSKNTAYLQMNSLRAEDTAVYYCARHGYGALDYWGQGTLVTVSSASTKGPSVFPLAPSSKSTSGGTAALGCLVKDYFPEPVTVSWNSGALTSGVHTFPAVLQSSGLYSLSSVVTVPSSSLGTQTYICNVNHKPSNTKVDKKVEPKSCDKTHTCPPCPAPEAAGGPSVFLFPPKPKDTLMISRTPEVTCVVVDVSHEDPEVKFNWYVDGVEVHNAKTKPREEQYNSTYRVVSVLTVLHQDWLNGKEYKCKVSNKALPASIEKTISKAKGQPREPQVYTLPPSREEMTKNQVSLTCLVKGFYPSDIAVEWESNGQPENNYKTTPPVLDSDGSFFLYSKLTVDKSRWQQGNVFSCSVMHEALHNHYTQKSLSLSPGKGGGGSGGGGSGGGGSGGGGSDIQMTQSPSSLSASVGDRVTITCRASQSVSSAVAWYQQKPGKAPKLLIYSASSLYSGVPSRFSGSRSGTDFTLTISSLQPEDFATYYCQQSSQFLITFGQGTKVEIKGGGGGEVQLVESGGGLVQPGGSLRLSCAASGFTLDSYYMHWVRQAPGKGLEWVASIAPYHGYTYYADSVKGRFTISADTSKNTAYLQMNSLRAEDTAVYYCARHGYGALDYWGQGTLVTVSS

SEQ ID NO: 30 - protein, 716 aa, synthetic construct
EVQLVESGGGLVQPGGSLRLSCAASGFTLDSYYMHWVRQAPGKGLEWVASIAPYHGYTYYADSVKGRFTISADTSKNTAYLQMNSLRAEDTAVYYCARHGYGALDYWGQGTLVTVSSASTKGPSVFPLAPSSKSTSGGTAALGCLVKDYFPEPVTVSWNSGALTSGVHTFPAVLQSSGLYSLSSVVTVPSSSLGTQTYICNVNHKPSNTKVDKKVEPKSCDKTHTGGGGSGGGGSGGGGSGGGGSDIQMTQSPSSLSASVGDRVTITCRASQSVSSAVAWYQQKPGKAPKLLIYSASSLYSGVPSRFSGSRSGTDFTLTISSLQPEDFATYYCQQSSQFLITFGQGTKVEIKGGGGGEVQLVESGGGLVQPGGSLRLSCAASGFTLDSYYMHWVRQAPGKGLEWVASIAPYHGYTYYADSVKGRFTISADTSKNTAYLQMNSLRAEDTAVYYCARHGYGALDYWGQGTLVTVSSGGGGSGGGGSEPKSSDKTHTCPPCPAPEAAGGPSVFLFPPKPKDTLMISRTPEVTCVVVDVSHEDPEVKFNWYVDGVEVHNAKTKPREEQYNSTYRVVSVLTVLHQDWLNGKEYKCKVSNKALPASIEKTISKAKGQPREPQVYTLPPSREEMTKNQVSLTCLVKGFYPSDIAVEWESNGQPENNYKTTPPVLDSDGSFFLYSKLTVDKSRWQQGNVFSCSVMHEALHNHYTQKSLSLSPGK

SEQ ID NO: 31 - protein, 692 aa, synthetic construct
EVQLVESGGGLVQPGGSLRLSCAASGFTLDSYYMHWVRQAPGKGLEWVASIAPYHGYTYYADSVKGRFTISADTSKNTAYLQMNSLRAEDTAVYYCARHGYGALDYWGQGTLVTVSSASTKGPSVFPLAPSSKSTSGGTAALGCLVKDYFPEPVTVSWNSGALTSGVHTFPAVLQSSGLYSLSSVVTVPSSSLGTQTYICNVNHKPSNTKVDKKVEPKSCDKTHTCPPCPAPEAAGGPSVFLFPPKPKDTLMISRTPEVTCVVVDVSHEDPEVKFNWYVDGVEVHNAKTKPREEQYNSTYRVVSVLTVLHQDWLNGKEYKCKVSNKALPASIEKTISKAKGQPREPQVYTLPPSREEMTKNQVSLTCLVKGFYPSDIAVEWESNGQPENNYKTTPPVLDSDGSFFLYSKLTVDKSRWQQGNVFSCSVMHEALHNHYTQKSLSLSPGKGGGGSGGGGSGGGGSGGGGSEVQLVESGGGLVQPGGSLRLSCAASGFTLDSYYMHWVRQAPGKGLEWVASIAPYHGYTYYADSVKGRFTISADTSKNTAYLQMNSLRAEDTAVYYCARHGYGALDYWGQGTLVTVSSASTKGPSVFPLAPSSKSTSGGTAALGCLVKDYFPEPVTVSWNSGALTSGVHTFPAVLQSSGLYSLSSVVTVPSSSLGTQTYICNVNHKPSNTKVDKKVEPKSCDKTHT

SEQ ID NO: 32 - protein, 692 aa, synthetic construct
EVQLVESGGGLVQPGGSLRLSCAASGFTLDSYYMHWVRQAPGKGLEWVASIAPYHGYTYYADSVKGRFTISADTSKNTAYLQMNSLRAEDTAVYYCARHGYGALDYWGQGTLVTVSSASTKGPSVFPLAPSSKSTSGGTAALGCLVKDYFPEPVTVSWNSGALTSGVHTFPAVLQSSGLYSLSSVVTVPSSSLGTQTYICNVNHKPSNTKVDKKVEPKSCDKTHTGGGGSGGGGSGGGGSGGGGSEVQLVESGGGLVQPGGSLRLSCAASGFTLDSYYMHWVRQAPGKGLEWVASIAPYHGYTYYADSVKGRFTISADTSKNTAYLQMNSLRAEDTAVYYCARHGYGALDYWGQGTLVTVSSASTKGPSVFPLAPSSKSTSGGTAALGCLVKDYFPEPVTVSWNSGALTSGVHTFPAVLQSSGLYSLSSVVTVPSSSLGTQTYICNVNHKPSNTKVDKKVEPKSCDKTHTCPPCPAPEAAGGPSVFLFPPKPKDTLMISRTPEVTCVVVDVSHEDPEVKFNWYVDGVEVHNAKTKPREEQYNSTYRVVSVLTVLHQDWLNGKEYKCKVSNKALPASIEKTISKAKGQPREPQVYTLPPSREEMTKNQVSLTCLVKGFYPSDIAVEWESNGQPENNYKTTPPVLDSDGSFFLYSKLTVDKSRWQQGNVFSCSVMHEALHNHYTQKSLSLSPGK